European Patent Specification EP 3 891 302 B1, published April 16, 2025. Title: COMPOSITIONS AND METHODS FOR DETECTION OF CANDIDA AURIS. Applicant: F. Hoffmann-La Roche AG Roche Diagnostics GmbH Roche Molecular Systems, Inc. The sequence listing filed with the application follows.

SEQUENCE LISTING (12 sequences)

SEQ ID NO: 1 - DNA, 20 bp, Artificial Sequence
  CAUR001 forward primer
tgagcgtgatgtcttctcac

SEQ ID NO: 2 - DNA, 20 bp, Artificial Sequence
  CAUR003 forward primer
gagcgtgatgtcttctcacc

SEQ ID NO: 3 - DNA, 28 bp, Artificial Sequence
  CAUR005 forward primer
actgatttggattttaaaactaacccaa

SEQ ID NO: 4 - DNA, 24 bp, Artificial Sequence
  CAUR007 forward primer
aactaacccaacgttaagttcaac

SEQ ID NO: 5 - DNA, 21 bp, Artificial Sequence
  CAUR002 reverse primer
cctgatttgaggcgacaacaa

SEQ ID NO: 6 - DNA, 22 bp, Artificial Sequence
  CAUR004 reverse primer
cgtctgcaagtcatactacgta

SEQ ID NO: 7 - DNA, 22 bp, Artificial Sequence
  CAUR006 reverse primer
cgatgattcacgtctgcaagtc

SEQ ID NO: 8 - DNA, 15 bp, Artificial Sequence
  CAUR008 reverse primer
caacgccaccgcgaa

SEQ ID NO: 9 - DNA, 24 bp, Artificial Sequence
  CAUR101HQ6 probe
  misc_feature: 5` HEX-Thr
  misc_feature: 3` phosphate
  misc_feature (6)..(7): BHQ-2
cttcgcggtggcgttgcattcaca

SEQ ID NO: 10 - DNA, 23 bp, Artificial Sequence
  CAUR103HQ6 probe
  misc_feature: 5` HEX-Thr
  misc_feature: 3` phosphate
  misc_feature (6)..(7): BHQ-2
ttcgcggtggcgttgcattcaca

SEQ ID NO: 11 - DNA, 30 bp, Artificial Sequence
  CAUR105HQ10 probe
  misc_feature: 5` HEX-Thr
  misc_feature: 3` phosphate
  misc_feature (10)..(11): BHQ-2
acaacggatctcttggttctcgcatcgatg

SEQ ID NO: 12 - DNA, 27 bp, Artificial Sequence
  CAUR107HQ8 probe
  misc_feature: 5` HEX-Thr
  misc_feature: 3` phosphate
  misc_feature (8)..(9): BHQ-2
ctcgcatcgatgaagaacgcagcgaaa